European Patent Specification EP 3 606 325 B1, published September 4, 2024. Title: Rational Design of Microbial-Based Biotherapeutics. Applicant: Gusto Global, LLC. The sequence listing filed with the application follows.

SEQUENCE LISTING (21 sequences)

SEQ ID NO: 1 - DNA, 1521 bp, Dialister succinatiphilus DSM21274 16S rRNA gene
gacgaacgctggcggcgtgcttaacacatgcaagtcgaacgagaggacaagagaagcttgcttcttttggaatcgagtggcaaacgggtgagtaacacgtaaacaacctgccttcaggatggggacaacagacggaaacgactgctaataccgaatacgcttgggagaccgcatgatcttccaaggaaagggtggcctctacctgtaagctatcgcctgaagaggggtttgcgtctgattaggcagttggtgaggtaacggcccaccaaacctacgatcagtagccggtctgagaggatgaacggccacactggaactgagacacggtccagactcctacgggaggcagcagtggggaatcttccgcaatgggcgaaagcctgacggagcaacgccgcgtgagtgatgacggccttcgggttgtaaagctctgtgatcggggacgaacggtccgtaagctaataccttatggaagtgacggtacccgaatagcaagccacggctaactacgtgccagcagccgcggtaatacgtaggtggcaagcgttgtccggaattattgggcgtaaagcgcgcgcaggcggctttctaagtccatcttaaaagtgcggggcttaaccccgtgatgggatggaaactgggaagctggagtatcggagaggaaagtggaattcctagtgtagcggtgaaatgcgtagagattaggaagaacaccggtggcgaaggcgactttctggacgacaactgacgctgaggcgcgaaagcgtggggagcaaacaggattagataccctggtagtccacgccgtaaacgatgaatactaggtgtaggaggtatcgaccccttctgtgccggagctaacacaataagtattccgcctgggaagtacgatcgcaagattaaaactcaaaggaattgacgggggcccgcacaagcggtggagtatgtggtttaattcgacgcaacgcgaagaaccttaccaggtcttgacattgatcgccattcacagaaatgtgaagttctccttcgggagacgagaaaacaggtggtgcacggctgtcgtcagctcgtgtcgtgagatgttgggttaagtcccgcaacgagcgcaacccctatcttatgttaccagcacgttatggtggggactcatgagagaccgccgcggacaacgcggaggaaggtggggatgacgtcaagtcatcatgccccttatgacctgggctacacacgtactacaatgggtgtcaacaaagagaagcgaaaccgcgaggtggagcgaacctcaaaaacacacccccagttcagattgcaggctgcaacccgcctgcatgaagtaggaatcgctagtaatcgcgggtcagcataccgcggtgaatacgttcccgggccttgtacacaccgcccgtcacactatgagagtcggaaacacccgaagccggtgaggtaaccgcaaggagccagccgtcgaaggtggagctgatgattggagtgaagtcgtaacaaggtagccgtatcggaagg

SEQ ID NO: 2 - DNA, 1342 bp, Megamonas funiformis DSM19343 16S rRNA gene
ctttgacataagcttccgcttgaagatgagcttgcgtctgattagctagttggtgagggtaaaggcccaccaaggcgacgatcagtagccggtctgagaggatgaacggccacattgggactgagacacggcccagactcctacgggaggcagcagtggggaatcttccgcaatgggcgaaagcctgacggagcaacgccgcgtgaacgatgaaggtcttaggatcgtaaagttctgttgttagggacgaaggataaggattataatacagtctttgtttgacggtacctaacgaggaagccacggctaactacgtgccagcagccgcggtaatacgtaggcggcaagcgttgtccggaattattgggcgtaaagggagcgcaggcgggaaactaagcggatcttaaaagtgcggggctcaaccccgtgatggggtccgaactggttttcttgagtgcaggagaggaaagcggaattcccagtgtagcggtgaaatgcgtagatattgggaagaacaccagtggcgaaggcggctttctggactgtaactgacgctgaggctcgaaagctagggtagcgaacgggattagataccccggtagtcctagccgtaaacgatggatactaggtgtgggaggtatcgactccttccgtgccggagttaacgcaataagtatcccgcctggggagtacggccgcaaggttgaaactcaaaggaattgacgggggcccgcacaagcggtggagtatgtggtttaattcgacgcaacgcgaagaaccttaccaagacttgacattgattgaaagacttagagataagttccttctcttcggagaacaagaaaacaggtggtgcatggctgtcgtcagctcgtgtcgtgagatgttgggttaagtcccgcaacgagcgcaacccctatactatgttgccagcatttcggatgggaactcatagtagactgccgcggacaacgcggaggaaggcggggatgacgtcaagtcatcatgccccttacgtcttgggctacacacgtactacaatgggatgaacagagggaagcgaaatcgcgaggtggagcggatccctaaaagcatctctcagttcggattgtaggctgaaactcgcctacatgaagtcggaatcgctagtaatcgcaggtcagcatactgcggtgaatacgttcccgggccttgtacacaccgcccgtcacaccacgaaagtcattcacacccgaagccggctaagggcctatggtaccgaccgtctaaggtgggggcgatgattggggtgaagtcgtaacaaggtagccgtatcggaaggtgcggctggatcacctcctta

SEQ ID NO: 3 - DNA, 1518 bp, Megamonas hypermegale DSM1672 16S rRNA gene
cctggctcaggacgaacgctggcggcgtgcttaacacatgcaagtcgaacggggtgtttatttcggtaaacaccaagtggcgaacgggtgagtaacgcgtaagcaatctaccttcaagatggggacaacacttcgaaaggggtgctaataccgaatgaatgagagatgaccgcatggatatttctctaaaggaggcctctgaaaatgcttccgcttgaagatgagcttgcgtctgattagctagttggtgagggtaaaggcccaccaaggcgacgatcagtagccggtctgagaggatgaacggccacattgggactgagacacggcccagactcctacgggaggcagcagtggggaatcttccgcaatgggcgaaagcctgacggagcaacgccgcgtgaacgaagaaggtcttaggatcgtaaagttctgttgttaggggcgaagggcaacattttgaataagggtgttgtttgacggtacttaacgaggaagccacggctaactacgtgccagcagccgcggtaatacgtaggcggcaagcgttgtccggaattattgggcgtaaagggagcgcaggcgggaagttaagcggactttaaaagtgcggggctcaaccccgtgagggggtccgaactgactttcttgagtgcaggagagggaagcggaattcctagtgtagcggtgaaatgcgtagatattaggaagaacaccagtggcgaaggcggctttctggactgtaactgacgctgaggctcgaaagctagggtagcgaacgggattagataccccggtagtcctagccgtaaacgatggatactaggtgtgggaggtatcgaccccttccgtgccggagttaacgcaataagtatcccgcctggggagtacggccgcaaggttgaaactcaaaggaattgacgggggcccgcacaagcggtggagtatgtggtttaattcgacgcaacgcgaagaaccttaccaagacttgacatcgactgacgtagttagagataagtatttttacttcggtaaacaggaagacaggtggtgcatggctgtcgtcagctcgtgtcgtgagatgttgggttaagtcccgcaacgagcgcaacccctatactatgttgccagcacgtaaaggtgggaactcatagtagactgccgcggacaacgcggaggaaggcggggatgacgtcaagtcatcatgccccttacgtcttgggctacacacgtactacaatgggatgaacagagggaagcgaagtcgcgaggcagagcggaaccctaaaagcatctctcagttcggattgcaggctgaaactcgcctgcatgaagtcggaatcgctagtaatcgcaggtcagcatactgcggtgaatacgttcccgggccttgtacacaccgcccgtcacaccacgaaagtcattcacacccgaagccggctaagggccgaaaggaaccgaccgtcgaaggtgggggcgatgattggggtgaagtcgtaacaaggtagccgtatcggaagg

SEQ ID NO: 4 - DNA, 1439 bp, Acidaminococcus intestine DSM21505 16S rRNA gene
gcggagacttatttcggtaagttcttagtggcgaacgggtgagtaacgcgtgggcaacctgccctccagttggggacaacattccgaaagggatgctaataccgaatgtgctccctcctccgcatggaggagggaggaaagatggcctctgcttgcaagctatcgctggaagatgggcccgcgtctgattagctagttggtggggtaacggctcaccaaggcgatgatcagtagccggtctgagaggatgaacggccacattgggactgagacacggcccaaactcctacgggaggcagcagtggggaatcttccgcaatggacgaaagtctgacggagcaacgccgcgtgagtgatgaaggtcttcggattgtaaaactctgttgttagggacgaaagcaccgtgttcgaacaggtcatggtgttgacggtacctaacgaggaagccacggctaactacgtgccagcagccgcggtaatacgtaggtggcaagcgttgtccggaattattgggcgtaaagagcatgtaggcgggcttttaagtctgacgtgaaaatgcggggcttaaccccgtatggcgttggatactggaagtcttgagtgcaggagaggaaaggggaattcccagtgtagcggtgaaatgcgtagatattgggaggaacaccagtggcgaaggcgcctttctggactgtgtctgacgctgagatgcgaaagccagggtagcaaacgggattagataccccggtagtcctggccgtaaacgatggatactaggtgtaggaggtatcgaccccttctgtgccggagttaacgcaataagtatcccgcctggggactacgatcgcaagattgaaactcaaaggaattgacgggggcccgcacaagcggtggagtatgtggtttaattcgacgcaacgcgaagaaccttaccaaggcttgacattgagtgaaagacctagagataggtccctcccttcggggacacgaaaacaggtggtgcatggctgtcgtcagctcgtgtcgtgagatgttgggttaagtcccgcaacgagcgcaacccctatcctatgttaccagcgcgtaatggcggggactcataggagactgccagggataacttggaggaaggcggggatgacgtcaagtcatcatgccccttatgtcttgggctacacacgtactacaatggtcggcaacaaagggcagcgaaaccgcgaggtggagcaaatcccagaaacccgaccccagttcggatcgtaggctgcaacccgcctacagtgaagttggaatcgctagtaatcgcaggtcagcatactgcggtgaatacgttcccgggccttgtacacaccgcccgtcacaccacgaaagttggtaacacccgaagccggtgagataaccttttaggagtcagctgtctaaggtggggccgatgattgggg

SEQ ID NO: 5 - DNA, 1478 bp, Bacteroides massiliensis DSM17679 16S rRNA gene
ggctcaggatgaacgctagctacaggcttaacacatgcaagtcgaggggcagcatggtcttagcttgctaaggccgatggcgaccggcgcacgggtgagtaacgcgtatccaacctgccttacactcttggacagccttctgaaagggagattaatacaagatgttatcatgagtaagcattttcgcatgattaaaggtttaccggtgtaagatggggatgcgttccattagatagtaggcggggtaacggcccacctagtcttcgatggataggggttctgagaggaaggtcccccacattggaactgagacacggtccaaactcctacgggaggcagcagtgaggaatattggtcaatggacgagagtctgaaccagccaagtagcgtgaaggatgaaggttctatggattgtaaacttcttttatacgggaataaacggatccacgtgtggatttttgcatgtaccgtatgaataaggatcggctaactccgtgccagcagccgcggtaatacggaggatccgagcgttatccggatttattgggtttaaagggagcgtagatgggttgttaagtcagttgtgaaagtttgcggctcaaccgtaaaattgcaattgatactggcagtcttgagtacagttgaggtaggcggaattcgtggtgtagcggtgaaatgcttagatatcacgaagaactccgattgcgaaggcagcttactaacctgtaactgacattgatgctcgaaagtgtgggtatcaaacaggattagataccctggtagtccacacggtaaacgatgaatactcgctgtaggcgatatacggtctgcggccaagcgaaagcattaagtattccacctggggagtacgccggcaacggtgaaactcaaaggaattgacgggggcccgcacaagcggaggaacatgtggtttaattcgatgatacgcgaggaaccttacccgggcttaaattgcaaccgaatatggcggaaacgctatagctagcaatagcggttgtgaaggtgctgcatggttgtcgtcagctcgtgccgtgaggtgtcggcttaagtgccataacgagcgcaacccttgccgatagttactaacaggtcatgctgaggactctgtcgggactgccatcgtaagatgtgaggaaggtggggatgacgtcaaatcagcacggcccttacgtccggggctacacacgtgttacaatggggggtacagagggctgctaccacgcaagtggatgccaatcccaaaaacctctctcagttcggattgaagtctgcaacccgacttcatgaagctggattcgctagtaatcgcgcatcagccacggcgcggtgaatacgttcccgggccttgtacacaccgcccgtcaagccatgggagccgggggtacctgaagtgcgtaaccgcaaggagcgccctagggtaaaactggtgactggggctaagtcgtaacaaggtaacc

SEQ ID NO: 6 - DNA, 1476 bp, Bacteroides stercoris ATCC43183 / DSM19555 16S rRNA gene
tggctcaggatgaacgctagctacaggcttaacacatgcaagtcgaggggcagcatcatcaaagcttgctttgatggatggcgaccggcgcacgggtgagtaacacgtatccaacctgccgacaacactgggatagcctttcgaaagaaagattaataccggatggcatagttttcccgcatgggatgattattaaagaatttcggttgtcgatggggatgcgttccattaggcagttggcggggtaacggcccaccaaacctacgatggataggggttctgagaggaaggtcccccacattggaactgagacacggtccaaactcctacgggaggcagcagtgaggaatattggtcaatggacgagagtctgaaccagccaagtagcgtgaaggatgactgccctatgggttgtaaacttcttttatacgggaataaagtgagccacgtgtggctttttgtatgtaccgtatgaataaggatcggctaactccgtgccagcagccgcggtaatacggaggatccgagcgttatccggatttattgggtttaaagggagcgtaggcgggttgttaagtcagttgtgaaagtttgcggctcaaccgtaaaattgcagttgatactggcgaccttgagtgcaacagaggtaggcggaattcgtggtgtagcggtgaaatgcttagatatcacgaagaactccgattgcgaaggcagcttactggattgtaactgacgctgatgctcgaaagtgtgggtatcaaacaggattagataccctggtagtccacacagtaaacgatgaatactcgctgttggcgatatacagtcagcggccaagcgaaagcattaagtattccacctggggagtacgccggcaacggtgaaactcaaaggaattgacgggggcccgcacaagcggaggaacatgtggtttaattcgatgatacgcgaggaaccttacccgggcttaaattgcaactgactgaatcggaaacggttctttcttcggacagttgtgaaggtgctgcatggttgtcgtcagctcgtgccgtgaggtgtcggcttaagtgccataacgagcgcaacccttacgggtagttaccatcaggttatgctggggactctacccggactgccgtcgtaagatgtgaggaaggtggggatgacgtcaaatcagcacggcccttacgtccggggctacacacgtgttacaatggggggtacagaaggcagctacacggcgacgtggtgctaatcccgaaagcctctctcagttcggattggagtctgcaacccgactccatgaagctggattcgctagtaatcgcgcatcagccacggcgcggtgaatacgttcccgggccttgtacacaccgcccgtcaagccatgaaagccgggggtacctgaagtacgtaaccgcgaggagcgtcctagggtaaaactggtgattggggctaagtcgtaacaaggtaacc

SEQ ID NO: 7 - DNA, 1484 bp, Barnesiella intestinihominis DSM21032 16S rRNA gene
gatgaacgctagcgacaggcctaacacatgcaagtcgaggggcagcggggaggtagcaatacctttgccggcgaccggcgcacgggtgagtaacacgtatgcaatccacctgtaacagggggataacccggagaaatccggactaataccccataatatgggcgctccgcatggagagttcattaaagagagcaattttggttacagacgagcatgcgctccattagccagttggcggggtaacggcccaccaaagcgacgatggataggggttctgagaggaaggtcccccacattggaactgagacacggtccaaactcctacgggaggcagcagtgaggaatattggtcaatggtcggcagactgaaccagccaagtcgcgtgagggaagacggccctacgggttgtaaacctcttttgtcggagagtaaagtacgctacgtgtagcgtattgcaagtatccgaagaaaaagcatcggctaactccgtgccagcagccgcggtaatacggaggatgcgagcgttatccggatttattgggtttaaagggtgcgtaggcggcacgccaagtcagcggtgaaatttccgggctcaacccggagtgtgccgttgaaactggcgagctagagtacacaagaggcaggcggaatgcgtggtgtagcggtgaaatgcatagatatcacgcagaaccccgattgcgaaggcagcctgctagggtgaaacagacgctgaggcacgaaagcgtgggtatcgaacaggattagataccctggtagtccacgcagtaaacgatgaatactaactgtttgcgatacaatgtaagcggtacagcgaaagcgttaagtattccacctggggagtacgccggcaacggtgaaactcaaaggaattgacgggggcccgcacaagcggaggaacatgtggtttaattcgatgatacgcgaggaaccttacccgggctcaaacgcagggggaatgtcggtgaaagccggcagctagtaatagtcacctgcgaggtgctgcatggttgtcgtcagctcgtgccgtgaggtgtcggcttaagtgccataacgagcgcaacccctatcgacagttactaacgggtgaagccgaggactctgtcgagactgccggcgcaagccgcgaggaaggtggggatgacgtcaaatcagcacggcccttacgtccggggcgacacacgtgttacaatggcaggtacagaaggcagccagtcagcaatgacgcgcgaatcccgaaaacctgtctcagttcggattggagtctgcaacccgactccatgaagctggattcgctagtaatcgcgcatcagccatggcgcggtgaatacgttcccgggccttgtacacaccgcccgtcaagccatggaagccgggagtacctgaagcatgcaaccgcaaggagcgtacgaaggtaataccggtaactggggctaagtcgtaacaaggtagccgtaccggaagg

SEQ ID NO: 8 - DNA, 1462 bp, Faecalibacterium prausnitzii DSM17677 16S rRNA gene
gatcctggctcaggcgaacgctggcggcgcgcctaacacatgcaagtcgaacgagcgagagagagcttgctttctcaagcgagtggcgaacgggtgagtaacgcgtgaggaacctgcctcaaagagggggacaacagttggaaacgactgctaataccgcataagcccacgacccggcatcgggtagagggaaaaggagcaatccgctttgagatggcctcgcgtccgattagctagttggtgaggtaacggcccaccaaggcgacgatcggtagccggactgagaggttgaacggccacattgggactgagacacggcccagactcctacgggaggcagcagtggggaatattgcacaatgggggaaaccctgatgcagcgacgccgcgtggaggaagaaggtcttcggattgtaaactcctgttgttgaggaagataatgacggtactcaacaaggaagtgacggctaactacgtgccagcagccgcggtaaaacgtaggtcacaagcgttgtccggaattactgggtgtaaagggagcgcaggcgggaaggcaagttggaagtgaaatccatgggctcaacccatgaactgctttcaaaactgtttttcttgagtagtgcagaggtaggcggaattcccggtgtagcggtggaatgcgtagatatcgggaggaacaccagtggcgaaggcggcctactgggcaccaactgacgctgaggctcgaaagtgtgggtagcaaacaggattagataccctggtagtccacactgtggccgatgtttactaggtgttggaggattgaccccttcagtgccgcagttaacacaataagtaatccacctggggagtacgaccgcaaggttgaaactcaaaggaattgacgggggcccgcacaagcagtggagtatgtggtttaattcgacgcaacgcgaagaaccttaccaagtcttgacatcctgcgacgcacatagaaatatgtgtttccttcgggacgcagagacaggtggtgcatggttgtcgtcagctcgtgtcgtgagatgttgggttaagtcccgcaacgagcgcaacccttatggtcagttactacgcaagaggactctggccagactgccgttgacaaaacggaggaaggtggggatgacgtcaaatcatcatgccctttatgacttgggctacacacgtactacaatggcgttaaacaaagagaagcaagaccgcgaggtggagcaaaactcagaaacaacgtcccagttcggactgcaggctgcaactcgcctgcacgaagtcggaattgctagtaatcgcagatcagcatgctgcggtgaatacgttcccgggccttgtacacaccgcccgtcacaccatgagagccggggggacccgaagtcggtagtctaaccgcaaggaggacgccgccgaaggtaaaactggtgattggggtgaagtcgtaacaaggtac

SEQ ID NO: 9 - DNA, 1428 bp, Subdoligranulum variabile DSM15176 16S rRNA gene
  misc_feature (1189)..(1189): n is a, c, g, or t
tgcaagtcgaacggagttatttcggttgaagttttcggatggatactggtttaacttagtggcgaacgggtgagtaacgcgtgagtaacctgccctggagtgggggacaacagttggaaacgactgctaataccgcataagcccacgatccggcatcggattgagggaaaaggatttattcgcttcaggatggactcgcgtccaattagctagttggtgaggtaacggcccaccaaggcgacgattggtagccggactgagaggttgaacggccacattgggactgagacacggcccagactcctacgggaggcagcagtgggggatattgcacaatgggggaaaccctgatgcagcgacgccgcgtggaggaagaaggttttcggattgtaaactcctgtcgttagggacgaatcttgacggtacctaacaagaaagcaccggctaactacgtgccagcagccgcggtaaaacgtagggtgcaagcgttgtccggaattactgggtgtaaagggagcgcaggcggaccggcaagttggaagtgaaatctatgggctcaacccataaattgctttcaaaactgctggccttgagtagtgcagaggtaggtggaattcccggtgtagcggtggaatgcgtagatatcgggaggaacaccagtggcgaaggcgacctactgggcaccaactgacgctgaggctcgaaagcatgggtagcaaacaggattagataccctggtagtccatgccgtaaacgatgattactaggtgttggaggattgaccccttcagtgccgcagttaacacaataagtaatccacctggggagtacgaccgcaaggttgaaactcaaaggaattgacgggggcccgcacaagcagtggagtatgtggtttaattcgaagcaacgcgaagaaccttaccaggtcttgacatccgatgcatagtgcagagatgcatgaagtccttcgggacatcgagacaggtggtgcatggttgtcgtcagctcgtgtcgtgagatgttgggttaagtcccgcaacgagcgcaacccttattgccagttactacgcaagaggactctggcgagactgccgttgacaaaacggaggaaggtggggatgacgtcaaatcatcatgccctttatgacctgggctacacacgtactacaatggcgtttaacaaagagangcaagaccgcgaggtggagcaaaactcaaaaacaacgtctcagttcagattgcaggctgcaactcgcctgcatgaagtcggaattgctagtaatcgcggatcagcatgccgcggtgaatacgttcccgggccttgtacacaccgcccgtcacaccatgagagccgggggggacccgaagtcggtaagtaagtctaaccgcaaggaggacgccgccgaaggtaaaactggtgattgggtg

SEQ ID NO: 10 - DNA, 1456 bp, Anaerostipes caccae DSM14662 16S rRNA gene
gcgcttaatacatgtcaagtcgaacgaagcatttaggattgaagttttcggatggatttcctatatgactgagtggcggacgggtgagtaacgcgtggggaacctgccctatacagggggataacagctggaaacggctgctaataccgcataagcgcacagaatcgcatgattcagtgtgaaaagccctggcagtataggatggtcccgcgtctgattagctggttggtgaggtaacggctcaccaaggcgacgatcagtagccggcttgagagagtgaacggccacattgggactgagacacggcccaaactcctacgggaggcagcagtggggaatattgcacaatgggggtaaaccctgatgcagcgacgccgcgtgagtgaagaagtatttcggtatgtaaagctctatcagcagggaagaaaacagacggtacctgactaagaagccccggctaactacgtgccagcagccgcggtaatacgtagggggcaagcgttatccggaattactgggtgtaaagggtgcgtaggtggcatggtaagtcagaagtgaaagcccggggcttaaccccgggactgcttttgaaactgtcatgctggagtgcaggagaggtaagcggaattcctagtgtagcggtgaaatgcgtagatattaggaggaacaccagtggcgaaggcggcttactggactgtcactgacactgatgcacgaaagcgtggggagcaaacaggattagataccctggtagtccacgccgtaaacgatgaatactaggtgtcggggccgtagaggcttcggtgccgcagcaaacgcagtaagtattccacctggggagtacgttcgcaagaatgaaactcaaaggaattgacggggacccgcacaagcggtggagcatgtggtttaattcgaagcaacgcgaagaaccttacctggtcttgacatcccaatgaccgaaccttaaccggttttttctttcgagacattggagacaggtggtgcatggttgtcgtcagctcgtgtcgtgagatgttgggttaagtcccgcaacgagcgcaacccctatctttagtagccagcatttaaggtgggcactctagagagactgccagggataacctggaggaaggtggggacgacgtcaaatcatcatgccccttatggccagggctacacacgtgctacaatggcgtaaacaaagggaagcgaagtcgtgaggcgaagcaaatcccagaaataacgtctcagttcggattgtagtctgcaactcgactacatgaagctggaatcgctagtaatcgtgaatcagaatgtcacggtgaatacgttcccgggtcttgtacacaccgcccgtcacaccatgggagtcagtaacgcccgaagtcagtgacccaaccgcaaggagggagctgccgaaggtgggaccgataactggggtgaagtcgtaacaagg

SEQ ID NO: 11 - DNA, 1616 bp, Anaerostipes hadrus DSM 3319 / ATCC 29173 16S rRNA gene
tttgatcctggctcaggatgaacgctggcggcgtgcttaacacatgcaagtcgaacgaaacaccttatttgattttcttcggaactgaagatttggtgattgagtggcggacgggtgagtaacgcgtgggtaacctgccctgtacagggggataacagtcagaaatgactgctaataccgcataagaccacagcaccgcatggtgcaggggtaaaaactccggtggtacaggatggacccgcgtctgattagctggttggtgaggtaacggctcaccaaggcgacgatcagtagccggcttgagagagtgaacggccacattgggactgagacacggcccaaactcctacgggaggcagcagtggggaatattgcacaatgggggaaaccctgatgcagcgacgccgcgtgagtgaagaagtatctcggtatgtaaagctctatcagcagggaagaaaatgacggtacctgactaagaagccccggctaactacgtgccagcagccgcggtaatacgtagggggcaagcgttatccggaattactgggtgtaaagggtgcgtaggtggtatggcaagtcagaagtgaaaacccagggcttaactctgggactgcttttgaaactgtcagactggagtgcaggagaggtaagcggaattcctagtgtagcggtgaaatgcgtagatattaggaggaacatcagtggcgaaggcggcttactggactgaaactgacactgaggcacgaaagcgtggggagcaaacaggattagataccctggtagtccacgccgtaaacgatgaatactaggtgtcggggccgtaggggcttcggtgccgcagccaacgcagtaagtattccacctggggagtacgttcgcaagaatgaaactcaaaggaattgacggggacccgcacaagcggtggagcatgtggtttaattcgaagcaacgcgaagaaccttacctggtcttgacatccttctgaccggtccttaaccggacctttccttcgggacaggagagacaggtggtgcatggttgtcgtcagctcgtgtcgtgagatgttgggttaagtcccgcaacgagcgcaacccctatctttagtagccagcatataaggtgggcactctagagagactgccagggataacctggaggaaggtggggacgacgtcaaatcatcatgccccttatgaccagggctacacacgtgctacaatggcgtaaacagagggaagcagcctcgtgagagtgagcaaatcccaaaaataacgtctcagttcggattgtagtctgcaactcgactacatgaagctggaatcgctagtaatcgcgaatcagaatgtcgcggtgaatacgttcccgggtcttgtacacaccgcccgtcacaccatgggagtcagtaacgcccgaagtcagtgacccaaccgtaaggagggagctgccgaaggcgggaccgataactggggtgaagtcgtaacaaggtagccgtatcggaaggtgcggctggatcacctcctttctaatcccgcggccatggcggccgggagcatgcgacgtcgggcccaattcgccctatagtgagtcgtattacaattcactggccgtcgtttaaa

SEQ ID NO: 12 - DNA, 1492 bp, Clostridium symbiosum ATCC14940 16S rRNA gene
  misc_feature (66)..(66): n is a, c, g, or t
  misc_feature (199)..(199): n is a, c, g, or t
agagtttgatcctggctcaggatgaacgctggcggcgtgcctaacacatgcaagtcgaacgaagcnatttaacggaagttttcggatggaagttgaattgactgagtggcggacgggtgagtaacgcgtgggtaacctgccttgtactgggggacaacagttagaaatgactgctaataccgcataagcgcacagtatngcatgatacagtgtgaaaaactccggtggtacaagatggacccgcgtctgattagctagttggtaaggtaacggcttaccaaggcgacgatcagtagccgacctgagagggtgaccggccacattgggactgagacacggcccaaactcctacgggaggcagcagtggggaatattgcacaatgggcgaaagcctgatgcagcgacgccgcgtgagtgaagaagtatttcggtatgtaaagctctatcagcagggaagaaaatgacggtacctgactaagaagccccggctaactacgtgccagcagccgcggtaatacgtagggggcaagcgttatccggatttactgggtgtaaagggagcgtagacggtaaagcaagtctgaagtgaaagcccgcggctcaactgcgggactgctttggaaactgtttaactggagtgtcggagaggtaagtggaattcctagtgtagcggtgaaatgcgtagatattaggaggaacaccagtggcgaaggcgacttactggacgataactgacgttgaggctcgaaagcgtggggagcaaacaggattagataccctggtagtccacgccgtaaacgatgaatactaggtgttggggagcaaagctcttcggtgccgtcgcaaacgcagtaagtattccacctggggagtacgttcgcaagaatgaaactcaaaggaattgacggggacccgcacaagcggtggagcatgtggtttaattcgaagcaacgcgaagaaccttaccaggtcttgacatcgatccgacgggggagtaacgtccccttcccttcggggcggagaagacaggtggtgcatggttgtcgtcagctcgtgtcgtgagatgttgggttaagtcccgcaacgagcgcaacccttattctaagtagccagcggttcggccgggaactcttgggagactgccagggataacctggaggaaggtggggatgacgtcaaatcatcatgccccttatgatctgggctacacacgtgctacaatggcgtaaacaaagagaagcaagaccgcgaggtggagcaaatctcaaaaataacgtctcagttcggactgcaggctgcaactcgcctgcacgaagctggaatcgctagtaatcgcgaatcagaatgtcgcggtgaatacgttcccgggtcttgtacacaccgcccgtcacaccatgggagtcagtaacgcccgaagtcagtgacccaaccgcaaggagggagctgccgaaggcgggaccgataactggggtgaagtcgtaacaaggtaacc

SEQ ID NO: 13 - DNA, 1498 bp, Clostridium boltea ATCC BAA-613 16S rRNA gene
agagtttgatcctggctcaggatgaacgctggcggcgtgcctaacacatgcaagtcgaacgaagcaattaaaatgaagttttcggatggatttttaattgactgagtggcggacgggtgagtaacgcgtggataacctgcctcacactgggggataacagttagaaatgactgctaataccgcataagcgcacagtgccgcatggtacagtgtgaaaaactccggtggtgtgagatggatccgcgtctgattagccagttggcggggtaacggcccaccaaagcgacgatcagtagccgacctgagagggtgaccggccacattgggactgagacacggcccaaactcctacgggaggcagcagtggggaatattgcacaatgggcgaaagcctgatgcagcgacgccgcgtgagtgaagaagtatttcggtatgtaaagctctatcagcagggaagaaaatgacggtacctgactaagaagccccggctaactacgtgccagcagccgcggtaatacgtagggggcaagcgttatccggatttactgggtgtaaagggagcgtagacggcgaagcaagtctgaagtgaaaacccagggctcaaccctgggactgctttggaaactgttttgctagagtgtcggagaggtaagtggaattcctagtgtagcggtgaaatgcgtagatattaggaggaacaccagtggcgaaggcggcttactggacgataactgacgttgaggctcgaaagcgtggggagcaaacaggattagataccctggtagtccacgccgtaaacgatgaatgctaggtgttggggggcaaagcccttcggtgccgtcgcaaacgcagtaagcattccgcctggggagtacgttcgcaagaatgaaactcaaaggaattgacggggacccgcacaagcggtggagcatgtggtttaattcgaagcaacgcgaagaaccttaccaagtcttgacatcctcttgaccggcgtgtaacggcgccttcccttcggggcaagagagacaggtggtgcatggttgtcgtcagctcgtgtcgtgagatgttgggttaagtcccgcaacgagcgcaacccttatccttagtagccagcaggtagagctgggcactctagggagactgccagggataacctggaggaaggtggggatgacgtcaaatcatcatgccccttatgatttgggctacacacgtgctacaatggcgtaaacaaagggaagcaaggcagtgatgtggagcaaatcccaaaaataacgtcccagttcggactgtagtctgcaacccgactacacgaagctggaatcgctagtaatcgcgaatcagaatgtcgcggtgaatacgttcccgggtcttgtacacaccgcccgtcacaccatgggagtcagcaacgcccgaagtcagtgacccaactcgcaagagagggagctgccgaaggcggggcaggtaactggggtgaagtcgtaacaaggtaaccgta

SEQ ID NO: 14 - DNA, 1427 bp, Blautia producta DSM2950 16S rRNA gene
tatcctggctcaggatgaacgctggcggcgtgcttaacacatgcaagtcgagcgaagcactaagacagatttcttcggattgaagcctttgtgactgagcggcggacgggtgagtaacgcgtgggtagcctacctcatacagggggataacagttagaaatgactgctaataccgcataagcgcacaggaccgcatggtctggtgtgaaaaactccggtggtatgagatggacccgcgtctgattagctagttggaggggtaacggcccaccaaggcgacgatcagtagccggcctgagagggtgaacggccacattgggactgagacacggcccagactcctacgggaggcagcagtggggaatattgcacaatggggggaaccctgatgcagcgacgccgcgtgaaggaagaagtatctcggtatgtaaacttctatcagcagggaagaaaatgacggtacctgactaagaagccccggctaactacgtgccagcagccgcggtaatacgtagggggcaagcgttatccggatttactgggtgtaaagggagcgtagacggaagagcaagtctgatgtgaaaggctggggcttaaccccaggactgcattggaaactgttgttctagagtgccggagaggtaagcggaattcctagtgtagcggtgaaatgcgtagatattaggaggaacaccagtggcgaaggcggcttactggacggtaactgacgttgaggctcgaaagcgtggggagcaaacaggattagataccctggtagtccacgccgtaaacgatgaatactaggtgtcgggtggctaagccattcggtgccgcagcaaacgcaataagtattccacctggggagtacgttcgcaagaatgaaactcaaaggaattgacggggacccgcacaagcggtggagcatgtggtttaattcgaagcaacgcgaagaaccttaccaagtcttgacatccctctgaccgycccgtaacggggrtttcccttcggggcagaggagacaggtggtgcatggttgtcgtcagctcgtgtcgtgagatgttgggttaagtcccgcaacgagcgcaacccttatccttagtagccagcayatgatggtgggcactctagggagactgccggggataacccgagggaaggcggggacgacgtcaaatcatcatgccccttatgatttgggctacacacgtgctacaatggcgtaaacaaagggaagcgagacagcgatgttgagcgaatcccaaaaataacgtcccagttcggactgcagtctgcaactcgactgcacgaagctggaatcgctagtaatcgcggatcagaatgccgcggtgaatacgttcccgggtcttgtacacaccgcccgtcacaccatgggagtcagtaacgcccgaagtcagtgacctaaccga

SEQ ID NO: 15 - DNA, 1458 bp, Blautia hydrogenotrophica DSM 10507 16S rRNA gene
  misc_feature (1416)..(1416): n is a, c, g, or t
gatgaacgctggcggcgtgcttaacacatgcaagtcgaacgaagcgatagagaacggagatttcggttgaagttttctattgactgagtggcggacgggtgagtaacgcgtgggtaacctgccctatacagggggataacagttagaaatgactgctaataccgcataagcgcacagcttcgcatgaagcggtgtgaaaaactgaggtggtataggatggacccgcgttggattagctagttggtgaggtaacggcccaccaaggcgacgatccatagccggcctgagagggtgaacggccacattgggactgagacacggcccaaactcctacgggaggcagcagtggggaatattgcacaatgggggaaaccctgatgcagcgacgccgcgtgaaggaagaagtatctcggtatgtaaacttctatcagcagggaagaaagtgacggtacctgactaagaagccccggctaattacgtgccagcagccgcggtaatacgtaaggggcaagcgttatccggatttactgggtgtaaagggagcgtagacggtttggcaagtctgatgtgaaaggcatgggctcaacctgtggactgcattggaaactgtcagacttgagtgccggagaggcaagcggaattcctagtgtagcggtgaaatgcgtagatattaggaggaacaccagtggcgaaggcggcctgctggacggtaactgacgttgaggctcgaaagcgtggggagcaaacaggattagataccctggtagtccacgctgtaaacgatgaatactaggtgtcgggtggcaaagccattcggtgccgcagcaaacgcaataagtattcccacctggggagtacgttcgcaagaatgaaactcaaaggaattgacggggacccgcacaagcggtggagcatgtggtttaattcgaagcaacgcgaagaaccttaccaaatcttgacatccctctgaccgggaagtaatgttcccttttcttcggaacagaggagacaggtggtgcatggttgtcgtcagctcgtgtcgtgagatgttgggttaagtcccgcaacgagcgcaacccttattcttagtagccagcaggtagagctgggcactctagggagactgccagggataacctggaggaaggtggggatgacgtcaaatcatcatgccccttatgatttgggctacacacgtgctacaatggcgtaaacaaagggaagcgaaggggtgacctggagcaaatctcaaaaataacgtctcagttcggattgtagtctgcaactcgactacatgaagctggaatcgctagtaatcgcgaatcagaatgtcgcggtgaatacgttcccgggtcttgtacacaccgcccgtcacaccatgggagtcagtaacgcccgaagtcagtgacccaaccnaaaggagggagctgccgaaggtgggactgataactggggtga

SEQ ID NO: 16 - DNA, 1456 bp, Marvinbryantia formatexigens DSM14469 16S rRNA gene
tggcggcgtgcttaacacatgcaagtcgagcgaagcattttaaatgaagttttcggacggaatttaaaatgactgagcggcggacgggtgagtaacgcgtggataacctgccttatacagggggataacagccagaaatggctgctaataccgcataagcgcacggtaccgcatggtacagtgtgaaaaactccggtggtataagatgggtccgcgttggattaggcagttggcggggtaaaggcccaccaaaccgacgatccatagccggcctgagagggtggacggccacattgggactgagacacggcccagactcctacgggaggcagcagtggggaatattgcacaatgggggaaaccctgatgcagcgacgccgcgtgggtgaagaagtatttcggtatgtaaagccctatcagcagggaagaaaatgacggtacctgaccaagaagccccggctaactacgtgccagcagccgcggtaatacgtagggggcaagcgttatccggatttactgggtgtaaagggagcgtagacggccatgcaagtctggtgtgaaaggcgggggctcaacccccggactgcattggaaactgtatggcttgagtgccggagaggtaagcggaattcctggtgtagcggtgaaatgcgtagatatcaggaggaacaccagtggcgaaggcggcttactggacggtaactgacgttgaggctcgaaagcgtggggagcaaacaggattagataccctggtagtccacgccgtaaacgatgaataccaggtgtcgggggacacggtccttcggtgccgcagcaaacgcactaagtattccacctggggagtacgttcgcaagaatgaaactcaaaggaattgacggggacccgcacaagcggtggagcatgtggtttaattcgaagcaacgcgaagaaccttaccaggtcttgacatccggacgaccggacagtaacgtgtccttcccttcggggcgtccgagacaggtggtgcatggttgtcgtcagctcgtgtcgtgagatgttgggttaagtcccgcaacgagcgcaacccctgttcccagtagccagcattcaggatgggcactctggggagactgccagggataacctggaggaaggcggggatgacgtcaaatcatcatgccccttatgatctgggctacacacgtgctacaatggcgtgaacagagggaagcgaacccgcgagggggagcaaatcccagaaataacgtcccagttcggattgtagtctgcaacccggctacatgaagctggaatcgctagtaatcgcggatcagcatgccgcggtgaatacgttcccgggtcttgtacacaccgcccgtcacaccatgggagtcggaaatgcccgaagtcagtgacccaaccggaaggagggagctgccgaaggcggggccggtaactggggtgaagtcgtaacaa

SEQ ID NO: 17 - DNA, 1529 bp, Clostridium scindens ATCC35704 16S rRNA gene
gagagtttgatcctggctcaggatgaacgctggcggcgtgcctaacacatgcaagtcgaacgaagcgcctggccccgacttcttcggaacgaggagccttgcgactgagtggcggacgggtgagtaacgcgtgggcaacctgccttgcactgggggataacagccagaaatggctgctaataccgcataagaccgaagcgccgcatggcgcggcggccaaagccccggcggtgcaagatgggcccgcgtctgattaggtagttggcggggtaacggcccaccaagccgacgatcagtagccgacctgagagggtgaccggccacattgggactgagacacggcccagactcctacgggaggcagcagtggggaatattgcacaatgggggaaaccctgatgcagcgacgccgcgtgaaggatgaagtatttcggtatgtaaacttctatcagcagggaagaagatgacggtacctgactaagaagccccggctaactacgtgccagcagccgcggtaatacgtagggggcaagcgttatccggatttactgggtgtaaagggagcgtagacggcgatgcaagccagatgtgaaagcccggggctcaaccccgggactgcatttggaactgcgtggctggagtgtcggagaggcaggcggaattcctagtgtagcggtgaaatgcgtagatattaggaggaacaccagtggcgaaggcggcctgctggacgatgactgacgttgaggctcgaaagcgtggggagcaaacaggattagataccctggtagtccacgccgtaaacgatgactactaggtgtcgggtggcaaggccattcggtgccgcagcaaacgcaataagtagtccacctggggagtacgttcgcaagaatgaaactcaaaggaattgacggggacccgcacaagcggtggagcatgtggtttaattcgaagcaacgcgaagaaccttacctgatcttgacatcccgatgccaaagcgcgtaacgcgctctttcttcggaacatcggtgacaggtggtgcatggttgtcgtcagctcgtgtcgtgagatgttgggttaagtcccgcaacgagcgcaacccctatcttcagtagccagcattttggatgggcactctggagagactgccagggagaacctggaggaaggtggggatgacgtcaaatcatcatgccccttatgaccagggctacacacgtgctacaatggcgtaaacaaagggaggcgaacccgcgagggtgggcaaatcccaaaaataacgtctcagttcggattgtagtctgcaactcgactacatgaagttggaatcgctagtaatcgcgaatcagaatgtcgcggtgaatacgttcccgggtcttgtacacaccgcccgtcacaccatgggagtcagtaacgcccgaagccggtgacccaacccgtaagggagggagccgtcgaaggtgggaccgataactggggtgaagtcgtaacaaggtagccgtatcggaaggtgcggctggatcacctccttc

SEQ ID NO: 18 - DNA, 1433 bp, Akkermansia muciniphila ATCC BAA-835 rRNA gene
aacgaacgctggcggcgtggataagacatgcaagtcgaacgagagaattgctagcttgctaataattctctagtggcgcacgggtgagtaacacgtgagtaacctgcccccgagagcgggatagccctgggaaactgggattaataccgcatagtatcgaaagattaaagcagcaatgcgcttggggatgggctcgcggcctattagttagttggtgaggtaacggctcaccaaggcgatgacgggtagccggtctgagaggatgtccggccacactggaactgagacacggtccagacacctacgggtggcagcagtcgagaatcattcacaatgggggaaaccctgatggtgcgacgccgcgtgggggaatgaaggtcttcggattgtaaacccctgtcatgtgggagcaaattaaaaagatagtaccacaagaggaagagacggctaactctgtgccagcagccgcggtaatacagaggtctcaagcgttgttcggaatcactgggcgtaaagcgtgcgtaggctgtttcgtaagtcgtgtgtgaaaggcgcgggctcaacccgcggacggcacatgatactgcgagactagagtaatggagggggaaccggaattctcggtgtagcagtgaaatgcgtagatatcgagaggaacactcgtggcgaaggcgggttcctggacattaactgacgctgaggcacgaaggccaggggagcgaaagggattagatacccctgtagtcctggcagtaaacggtgcacgcttggtgtgcggggaatcgaccccctgcgtgccggagtaacgcgttaagcgtgccgcctggggagtacggtcgcaagattaaaactcaaagaaattgacggggacccgcacaagcggtggagtatgtggcttaattcgatgcaacgcgaagaaccttacctgggcttgacatgtaatgaacaacatgtgaaagcatgcgactcttcggaggcgttacacaggtgctgcatggccgtcgtcagctcgtgtcgtgagatgtttggttaagtccagcaacgagcgcaacccctgttgccagttaccagcacgtgaaggtggggactctggcgagactgcccagatcaactgggaggaaggtggggacgacgtcaggtcagtatggcccttatgcccagggctgcacacgtactacaatgcccagtacagagggggccgaagccgcgaggcggaggaaatcctaaaaactgggcccagttcggactgtaggctgcaacccgcctacacgaagccggaatcgctagtaatggcgcatcagctacggcgccgtgaatacgttcccgggtcttgtacacaccgcccgtcacatcatggaagctggtcgcacccgaagtatctgaagccaaccgcaaggaggcagggtcctaaggtgagactggtaactgggatg

SEQ ID NO: 19 - DNA, 1484 bp, Clostridium saccharogumia DSM17460 16S rRNA gene
aagagtttgatcctggctcaggatgaacgctggcggcgtgcctaatacatgcaagtcgaacgcgggcagtaatgtccgagtggcgaacgggtgagtaagacataagtaacctgccctttacagggggataactattggaaacgatagctaagaccgcataggtaaagataccgcatggtaggtttattaaaagtgccaaggcactggtagaggatggacttatggcgcattagctggttggtgaggtaacggctcaccaaggcgacgatgcgtagccgacctgagagggtgaccggccacactgggactgagacacggcccagactcctacgggaggcagcagtagggaattttcggcaatggggggaaccctgaccgagcaacgccgcgtgaaggaggaaggtcttcggactgtaaacttctgttataaaggaagaaaggcggatacagggaatggtatccgagtgacggtactttatgaggaagccacggctaactacgtgccagcagccgcggtaatacgtaggtggcaagcgttatccggaattattgggcgtaaagagggagcaggcggcagcaagggtctgtggtgaaagactgaagcttaacttcagtaagccatagaaaccgggcagctagagtgcaggagaggatcgtggaattccatgtgtagcggtgaaatgcgtagatatatggaggaacaccagtggcgaaggcgacgatctggcctgcaactgacgctcagtcccgaaagcgtggggagcaaataggattagataccctagtagtccacgccgtaaacgatgagtactaagtgttgggagtcaaatctcagtgctgcagttaacgcagtaagtactccgcctgagtagtacgttcgcaagaatgaaactcaaaggaattgacgggggcccgcacaagcggtggagcatgtggtttaattcgaagcaacgcgaagaaccttaccaggtcttgacatactcataaaggctccagagatggagagataggtatatgggatacaggtggtgcatggttgtcgtcagctcgtgtcgtgagatgttgggttaagtcccgcaacgagcgcaacccttatcgttagttaccatcattaagttggggactctagcgagactgccagtgacaagctggaggaaggcggggatgacgtcaaatcatcatgccccttatgacctgggctacacacgtgctacaatggatggagcagagggaagcgaagccgcgaggtggagcgaaacccagaaaaccattctcagttcggattgtagtctgcaactcgactacatgaagttggaatcgctagtaatcgcgaatcagcatgtcgcggtgaatacgttctcgggccttgtacacaccgcccgtcacaccatgagagttgataacacccgaagccggtggcctaaccgcaaggagggagctgtctaaggtgggattgatgattggggtgaagtcgtaacaagggt

SEQ ID NO: 20 - DNA, 1519 bp, Clostridium ramosum DSM1402 16S rRNA gene
gagagtttgatcctggctcaggatgaacgctggcggcgtgcctaatacatgcaagtcgaacgcgagcacttgtgctcgagtggcgaacgggtgagtaatacataagtaacctgccctagacagggggataactattggaaacggatagctaagaccgcataggtacggacactgcatggtgaccgtattaaaagtgcctcaaagcactggtagaggatggacttatggcgcattagctggttggcggggtaacggcccaccaaggcgacgatgcgtagccgacctgagagggtgaccggccacactgggactgagacacggcccagactcctacgggaggcagcagtagggaattttcggcaatgggggaaaccctgaccgagcaacgccgcgtgaaggaagaaggttttcggattgtaaacttctgttataaagaagaacggcggctacaggaaatggtagccgagtgacggtactttattttagaaagccacggctaactacgtgccagcagccgcggtaatacgtaggtggcaagcgttatccggaattattgggcgtaaagagggagcaggcggcagcaagggtctgtggtgaaagcctgaagcttaacttcagtaagccatagaaaccaggcagctagagtgcaggagaggatcgtggaattccatgtgtagcggtgaaatgcgtagatatatggaggaacaccagtggcgaaggcgacgatctggcctgcaactgacgctcagtcccgaaagcgtggggagcaaataggattagataccctagtagtccacgccgtaaacgatgagtactaagtgttggatgtcaaagttcagtgctgcagttaacgcaataagtactccgcctgagtagtacgttcgcaagaatgaaactcaaaggaattgacgggggccgcacaagcggtggagcatgtggtttaattcgaagcaacgcgaagaaccttaccaggtcttgacatactcataaaggctccagagatggagagatagctatatgagatacaggtggtgcatggttgtcgtcagctcgtgtcgtgagatgttgggttaagtcccgcaacgagcgcaacccttatcgttagttaccatcattaagttggggactctagcgagactgccagtgacaagctggaggaaggcggggatgacgtcaaatcatcatgccccttatgacctgggctacacacgtgctacaatggatggtgcagagggaagcgaaccgcgaggtgaagcaaaacccataaaaaccattctcagttcggattgtagtctgcaactcgactacatgaagttggaatcgctagtaatcgcgaatcagcatgtcgcggtgaatacgttctcgggccttgtacacaccgcccgtcacaccacgagagttgataacacccgaagccggtggcctaaccgcaaggaaggagctgtctaaggtgggattgatgattggggtgaagtcgtaacaaggtatccctacgggaacgtgcggctggatcacctcc

SEQ ID NO: 21 - DNA, 1438 bp, Lactonifactor longoviformis DSM17459 16S rRNA gene
gagtttgattatggctcaggatgaacgctggcggcgtgcttaacacatgcaagtcgaacgaagcatatagagacgagtatttcggtatgagtaactatatgactgagtggcggacgggtgagtaacgcgtggataacctgcctcatacagggggataacagttagaaatgactgctaataccgcataagcgcacagtgctgcatggcacagtgtgaaaagctccggcggtatgagatggatccgcgtttgattagctagttggtggggtaaaggcctaccaaggcgacgatcaatagccgacctgagagggtgaccggccacattgggactgagacacggcccaaactcctacgggaggcagcagtggggaatattgcacaatgggggaaaccctgatgcagcgacgccgcgtgaaggaagaagtatttcggtatgtaaacttctatcagcagggaagaaaatgacggtacctgactaagaagccccggctaattacgtgccagcagccgcggtaatacgtaaggggcaagcgttatccggatttactgggtgtaaagggagcgtagacggcagtgcaagtctgatgtgaaagcccggggctcaaccccgggactgcattggaaactgtgcagctagagtgtcggagaggtaagtggaattcctagtgtagcggtgaaatgcgtagatattaggaggaacaccagtggcgaaggcggcttactggacgataactgacgttgaggctcgaaagcgtggggagcaaacaggattagataccctggtagtccacgccgtaaacgatgaatactaggtgtcgggcgccaaaggcgttcggtgccgcagcaaacgcaataagtattccacctggggagtacgttcgcaagaatgaaactcaaaggaattgacggggacccgcacaagcggtggagcatgtggtttaattcgaagcaacgcgaagaaccttaccaagtcttgacatctgcctgaccggtccgtaacaggacccttccttcgggacaggcaagacaggtggtgcatggttgtcgtcagctcgtgtcgtgagatgttgggttaagtcccgcaacgagcgcaacccttatccttagtagccagcaggtagagctgggcactctagggagactgccagggacaacctggaggaaggtggggatgacgtcaaatcatcatgccccttatgatttgggctacacacgtgctacaatggcgtaaacaaagggaagcgaaggggtgacctgaagcaaatcccaaaaataacgtctcagttcggattgtagtctgcaactcgactacatgaagctggaatcgctagtaatcgcgaatcagaatgtcgcggtgaatacgttcccgggtcttgtacacaccgcccgtcacaccatgggagtcggatatgcccgaagccggtgaccgaacccgaaa